European Patent Specification EP 4 225 930 B1, published May 14, 2025. Title: Process for the production of a filamentous fungus whole broth enzyme composition with low viscosity. Applicant: Clariant International Ltd. The sequence listing filed with the application follows.

SEQUENCE LISTING (30 sequences)

SEQ ID NO: 1 - DNA, 4572 bp, Trichoderma reesei
  Seq1 native gene
atgagggcctatcagatcgagatgctcgacaagagcctcaagcaaaatgtcattgttgctgtatgttgaagtttctctccaatcccccgtctccccctttgctgtcgttgtcttcgacgttgaaagacatgtccattgaccaaggggcgttgttataaatctagatggacacgggaagtggcaagactcaagtgtaagttgtgcatcttcatcatcggcagcccacgtaacctgtgccagcccttagcacccttcttcgcaaaagactgacttggcgcttgcatcagagctgtgcttcgtatcaagaaggagctggaaatctgcgatgcatcaaaggtgagtctgccgtctggatacagttgcacaacgacctggacagctgcactgacgcagcacgcatcagatcatctggttcatcgcgccaacagtttcgctgtgtcatcagcaacacgatgtgctcaagttgcagatacctgccgtgcccatgatgacactggccgggaactccaatatcgatgcttgggggccggatatctgggccattcttctcgacacggttcgaattgtcatatccacaccccaggttctgctcgatgcccttgaccatgcttacctgaacttgggtcttctggcgctgcttgtatttgatgaaggtatgggacgacctgccttcactctgtaaaggcaaaggggccgccagaagttgcaaatcgctgacgtgtcttgtgcaaaagtccacaactgcattggcagaagtccaggcggcaaaatcatgctccaccactaccatccgcgcaagctggctggtgaaagcgtgcctgctgttctgggtctgacggcaactccgagcattcagtctgagcttgccgatattgatgccttggaatggctgatggatgcaagatgcgtctcgcccactctccatcgcgacgaactgctcaaatgcgtcaagaggcccaatatcaagcacatcatctataaagccggcaaagaagacatcacgacgcccaccatgcgcgacttggatcgggtctaccgggcgctggacattctcgaagacccctacatactcatgctgcgcaacaaccctacggaccgaaacaaccgcctgctgctaacagccattgaaaagtacgatacctacacacagaaccagatgaagtcgttctgcgcccgatcaagagagatatgcaagcaactcggtccctgggctgctgacctcttcatctggaaggccatctcagctcacttggacaaggtggacaggcagacggatggagttgacgagtatggcaacaagtggtcgtcggggtcgacaagcttcctggaaaagaagcacctggccgacatctatcgtcgagtcaaggtccaacgtccttccgatgtgccacaggtctttgaagacatttccgacaaggtcggtaagctaatctttgagcttctgtcggtagaggagcccacggtgggcatcatcttcgtcgaggaacgagtcatggttgctatgctggccgaggttctctctgtcaaccacacaatcacgtcccggtaccggatcgggaccatggttggcacctcaaattacgctgggcggcggaaggccgtttatgacttcgaccagaaaacggactacaaggacctgcagagcttccgctccggcaagattaacctgctgattgcgacgtcagtgctggaggagggcatcgacgtgcctgcctgcaacctagtcatatgctttgacactccgacgaccccaaagtcctttatccagcggcgcggacgggctcgctccaaggactcgaatctccttcttttctttgacgatgccaaccctgcgatcttgaagtggcaggcgaaagaggaggagatgaacaggatcttcgaagacgaagagagggcgattcgcgaactcggcaaactggaagattcggagagtccgagcaccatctccttcaccgtcccgtctaccggcgcaaggctagattttgacaatgcgaagcagcacctcgagcacttctgcagagtcttgtgcccgtcggactttgtggacagccgcccggactacatcatccgcagggagcaggactctcctttgttgactgccattgtactgctccctccgtttctgccggtgaatctgaggcagcacaccagtgcttctccttggcgctccgagaagaacgccaccaaggatgctgcgtatcaggcgtatatagccctgtatgacgcgaagctcgtcaacgagaacctgctgcccttcaagtccagcgacatgctcggaatcgataagcgagtatccgaggtgccggtcgagccgttgatgaagccatggcatcgtgtcgctcctgcgtggcgggaagctggcgacaagtggctttactccttgagctgcgtggaggaggacggccgagtaagtgcagagtacgaggttctgctgccagtctggctgaaccagcctcagcccctgaaaatgttcctcgaccgcaatcaccaggtggagttgcagctgaaggccgggatacccgtgccgcacgagcaagttgcgtccctgccagatcatacatcgactttgctggcgctgcatttcggtcatcgatggcctctcgagcagaaagagcacgtcattcgggtctgggccaaggatcaacccctatcgctgaaccaaattggcgagctcacatacgatccacagaatgagagcgtcagccggggagagtttctcatccgggacaacaccagagccccctacctgtacaaggataccattgcgttcaagcccgaaccgagccaggtccagaataccttttacgagtacgacaaggcgcccgaagacgtgccgtatctcgtgctcaccaaatggacgcggcggaccgactttctgcatcgcctccaagggaatcccgccaagaatgaggttagtagcaagccatacgcacgcgtatatccgctgtcgtgggcgacagtcgataccatccccgccaggcacgcccagtttggcatgctgatcccgaccatgatccacgagctcggcgtcatgctcatggccaaggagctggcctactccgttctcgacgaggttggcatttcggatctgcagctggtcaaggaggccatcagcgcgcggagtgcctcggagccggtgaattacgagaggctggagtttttgggcgactcgattctcaagttttgtgcctgtatgcgcgccgctgctgaaagtaagttgctcaagcgttttactcatatatgactcctgtgtgcacctgtcctctgacatggaactgttttgctgaccacatttgatactgcctagaacccgactatcccgagggctatctctcgtattggagagaccgactcgtctccaactcgaggctgtacaaagccgctctcgagtttgggctgccgaggttcatcttgacgaaaccttttaccggtcaaaagtggcgcccactctacctggacgaggtcctccagcaaggggacgtcgctacgccggagaagagaaaattatcgaccaagacgctcgcagacgtggtcgaggcgctgatcggggcctcatacgtcgatggaggcctttcaaaggcagtgacttgcatctcaaaattcgtccccgaaggctcgtggaccagtgttgatgcagatagagagtctctctttgcgagagtgccagacggcgagcctctcccgccgccattggagccgctggagaagttgatcggctacacgttccagaaaaaggcgctcttgatggaggctctgacgcatgcctcgtatgctgcagacttcggaacgcgatctctcgagaggctcgaattcataggagacgctgtcctggacaacattatcgttacgaagctctttaggctgaagccagcgctgccccatttcaggatgcatacgctgaagacgggcctggtgaatggggactttcttgctttcatgacaatggagcacggagtgcaactggcggcggaccctgtggtgacagaagaagctacggtggaggtcccggaaacgatttcctacctgtggtcgtttttgaggcaggcctcttttcccattgccatcgagctgaaggagacgaacaagcggcacgctgccctgagagagcagattcacgaagcaatggacaatgacgatcattacccctgggcgctgctggccgccctgagcccgaagaagttctactctgacctcttcgaggcggttctcggcgctgtgtggatcgactccgggtcgctggcggcgtgcgagggcatggttgcgcagtttgggatcttaaagtacatggatcggctgctgcgtgacgaagtccacgtgcagcatcctaaggaggagctgggcatgtgggcaaacacagagactgtgacgtacgagctcgagatgaaggggagcgaggagagcgcgggggagagggagtatttctgcaaggtgtttgttggaaagagggaggttgtggaggttcgtgggggggtcaataaggaggaggtgaagacgaagggtgcgacggaggcgttgcggattttgagggaggagaaaaggcgcggtgctgaggatgtggtgatggtgggataa

SEQ ID NO: 2 - DNA, 3679 bp, Trichoderma reesei
  SEQ1 mutation flanks 1
gactgaaggccttcatcaaatacaagcagcgccagaagacccaagttcaggtaagcatggtcaagggcatcgagcagaacctggggtgtggatatgacaattcgaaccgtgtcgagaagaatggcccagatatccggcccccaagcatcgatattggagttcccggccagtgtcatcatgggcacggcaggtatctgcaacttgagcacatcgtgttgctgatgacacagcgaaactgttggcgcgatgaaccagatgatctgatgcgtgctgcgtcagtgcagctgtccaggtcgttgtgcaactgtatccagacggcagactcacctttgatgcatcgcagatttccagctccttcttgatacgaagcacagctctgatgcaagcgccaagtcagtcttttgcgaagaagggtgctaagggctggcacaggttacgtgggctgccgatgatgaagatgcacaacttacacttgagtcttgccacttcacgtgtccatctagatttataacaacgccccttggtcaatggacatgtctttcaacgtcgaagacaacgacagcaaagggggagacgggggattggagagaaacttcaacatacagcaacaatgacattttgcttgaggctcttgtcgagcatctcgatctgataggccctcatgactttgacttgctctccctcctcgcccagcagtgctgcctgggagcctgaggttgttgtcgggatggctccatcttgaccgggcgtaggctgcttgatatcagctccaggcacggcagcctcgtcggcgacatggccatcgggagcaccatccgaccccgtggccgcgcccgcccctttctcgacggcgtggccagtcacatagttgagcgatggagccacgtctccagaggagcaagacgaccatgaatccgcgtccgacgacgacgacgagcgtgggcgcacccgcggcacgtcatccccagcgctcgccaggcccggagcagcagccgaagcagcgcggacaggaccaggaccagacccaggccctgaccctgaccctgatggcagcccagggccagccgccgctactagctgcaacatggaaaggcgacggcggcagtttggcgctcccgcggcggcggatcccggggtgtgactcaggcagcggcccctgcgaagcacccgcagcctcagggagcgtattctgacgtgtcgggcagacgcaacgagtgcgtatcgagcgactagctgcgcgtgaatcccggctcgcgatgcctcacggcgacggcggcggagttggttgcggggttggcgactcgacgctggcgggctgggacgcggatttgcacctggatcacctggatctggagctggagctgctggattcatgcccctgctcggcgggaagccggtgatttgcgtggctgccactggggagctaagagagaggcaagccgtagtcttagtcgtagttatatgtagttgtaaggtaaggcaaggtacatgtagtcgtctgtagggcctgtctagcgaaccttgaggtttcctggatccacggcgagcttggccagcatcagagagaggaggaggaggcagagaggcgtcaacagctgaggcgtcacggctcgagtgtcacaggcatcgcttccccgcaggtggaacaaggcgtgtgtcctttcgttgggctgctgagatgccaattgcttgcttgctgggggtgagagagaggccgcagaggtgtaggaggaggagacgcaattgggtgacgtggggggagtgaatgaatacaacgtcaaagcaggactgcgaattcaatctatggcaggcaaggacactcgtgcacgacaggctacatagctactattagcaaacggaggatgttgtttttgtgttggttcatgcagccactcatgcagagccccggcctcttctcaccttgtttgggttgttgaagcttgtttcgtggcttgatagtgagccgctgcgttaagattcaaactgtcaccgttagcgtcggcagcctcgttcacggcctctccttggtttctggaactctcacaggtatgtcaagcaagaatgtaacaagacacagcccgggctcttgtctgttaccaggtcatatgagccagggatcaagaaatccgcggaaaggtcaataaaatgggagttactgagtatattccgtcccgtgccttttcttcatgctggtctctggaggaaatctcacggctatcgtcacgaatggccgaataagtgcgaccatcttcagagcttcgtgtgactggcgaccatctttacccgaagtcagatagacaggaatcaccattggtagcagtgactaattaatgcactgttacaacacatgactgacaagtttcgaaaaccaagaataaggtactatcaatatcataagtacctaggatctaaggtatgtaggcagaccgtcatcatcaccttcaaacccccgacaggacaggcctcaatccccggcagtaggtacatactctatctccgggacttgacgacccaccattgcgattgccgcctcaatgccagaaggaacttttgtcctcccagtgctttgtcctgctactgtcattaccaagcaagccttaggagtcataagagtcatactgaaccttaggtacttgttgggcagagccatgtggcctacactcccaaactcaaaattactggtccgttcatgccttggatcatgtatctttccatttgccaatcataggcctcccggaactttcaagcaatagagaggtcagctcgatgctggacagggcagaccgtacttacacgtacctaggtagcctctctgtagaacctttgaccctcaaaaggttcatcaccaagttattgcgtagcatgacctagaatactgaaattagatcgcgcaagtagcaataattcgctatactatgtatgcggcaagtcgcatttcagaagccggttctgttcaaccacagtccaaccgtcgtcaatctggagatgcgtcacaggagccgcaggtgactgcacagcgatgcaccgtggtgatgacattgaatctgcctaggtataattacctacattttcaatgtctgtcttcaaaaatagaataaagtgccacttggcattcgacaattgttgtgttgaacaattgggagtatctacgtcgtgaatcatgttgcaagcaagaggtataggtaggtaccttacctgttgaagcagctagcgccctagaggcagcctctgatgtcgtcttgtcattttttgatccatctcaaacaagtctcaacaacgcatcccatgcaccatggagcttttcgcaacaggcttcaacgcctggaaccagctcactttcaccaaaggcagcccccaagaggccatcccagaggaaccagatgacctcttcggctttacaaaagttctctccgccacatccattgaacggccagtatcgcgcctcacttacaccatcggtaccttatatcaaatcacaacctatctcataccccatcacacctcccttttacgccctataaaagaccattaccgcctaaacctcaacaatcaaaccacaaactgacaaaagatttcccccccctccagtccgaaaagacgaccacctcatcctcgccggccatggcccctcgcagcacaacctcgagcacctctacgcgtccgccgaaacgtttcgact

SEQ ID NO: 3 - DNA, 4112 bp, Trichoderma reesei
  SEQ1 mutation flanks 2
gactgaagtacttcatctggttctgtgtgtaggtatcgtacttttcaatggctgttagcagcaggcggttgtttcggtccgtagggttgttgcgcagcatgagtatgtaggggtcttcgagaatgtccagcgcccggtagacccgatccaagtcgcgcatggtgggcgtcgtgatgtcttctttgccggctttatagatgatgtgcttgatattgggcctcttgacgcatttgagcagttcgtcgcgatggagagtgggcgagacgcatcttgcatccatcagccattccaaggcatccaatatcggcaagctcagactgaatgctcggagttgccgtcagacccagaacagcaggcacgctttcaccagccagcttgcgcggatggtagtggtggagcatgattttgccgcctggacttctgccaatgcagttgtggacttttgcacaagacacgtcagcgatttgcaacttctggcggcccctttgcctttacagagtgaaggcaggtcgtcccataccttcatcaaatacaagcagcgccagaagacccaagttcaggtaagcatggtcaagggcatcgagcagaacctggggtgtggatatgacaattcgaaccgtgtcgagaagaatggcccagatatccggcccccaagcatcgatattggagttcccggccagtgtcatcatgggcacggcaggtatctgcaacttgagcacatcgtgttgctgatgacacagcgaaactgttggcgcgatgaaccagatgatctgatgcgtgctgcgtcagtgcagctgtccaggtcgttgtgcaactgtatccagacggcagactcacctttgatgcatcgcagatttccagctccttcttgatacgaagcacagctctgatgcaagcgccaagtcagtcttttgcgaagaagggtgctaagggctggcacaggttacgtgggctgccgatgatgaagatgcacaacttacacttgagtcttgccacttcccgtgtccatctagatttataacaacgccccttggtcaatggacatgtctttcaacgtcgaagacaacgacagcaaagggggagacgggggattggagagaaacttcaacatacagcaacaatgacattttgcttgaggctcttgtcgagcatctcgatctgataggccctcatgactttgacttgctctccctcctcgcccagcagtgctgcctgggagcctgaggttgttgtcgggatggctccatcttgaccgggcgtaggctgcttgatatcagctccaggcacggcagcctcgtcggcgacatggccatcgggagcaccatccgaccccgtggccgcgcccgcccctttctcgacggcgtggccagtcacatagttgagcgatggagccacgtctccagaggagcaagacgaccatgaatccgcgtccgacgacgacgacgagcgtgggcgcacccgcggcacgtcatccccagcgctcgccaggcccggagcagcagccgaagcagcgcggacaggaccaggaccagacccaggccctgaccctgaccctgatggcagcccagggccagccgccgctactagctgcaacatggaaaggcgacggcggcagtttggcgctcccgcggcggcggatcccggggtgtgactcaggcagcggcccctgcgaagcacccgcagcctcagggagcgtattctgacgtgtcgggcagacgcaacgagtgcgtatcgagcgactagctgcgcgtgaatcccggctcgcgatgcctcacggcgacggcggcggagttggttgcggggttggcgactcgacgctggcgggctgggacgcggatttgcacctggatcacctggatctggagctggagctgctggattcatgcccctgctcggcgggaagccggtgatttgcgtggctgccactggggagctaagagagaggcaagccgtagtcttagtcgtagttatatgtagttgtaaggtaaggcaaggtacatgtagtcgtctgtagggcctgtctagcgaaccttgaggtttcctggatccacggcgagcttggccagcatcagagagaggaggaggaggcagagaggcgtcaacagctgaggcgtcacggctcgagtgtcacaggcatcgcttccccgcaggtggaacaaggcgtgtgtcctttcgttgggctgctgagatgccaattgcttgcttgctgggggtgagagagaggccgcagaggtgtaggaggaggagacgcaattgggtgacgtggggggagtgaatgaatacaacgtcaaagcaggactgcgaattcaatctatggcaggcaaggacactcgtgcacgacaggctacatagctactattagcaaacggaggatgttgtttttgtgttggttcatgcagccactcatgcagagccccggcctcttctcaccttgtttgggttgttgaagcttgtttcgtggcttgatagtgagccgctgcgttaagattcaaactgtcaccgttagcgtcggcagcctcgttcacggcctctccttggtttctggaactctcacaggtatgtcaagcaagataacaagacacagcccgggctcttgtctgttaccaggtcatatgagccagggatcaagaaatccgcggaaaggtcaataaaatgggagttactgagtatattccgtcccgtgccttttcttcatgctggtctctggaggaaatctcacggctatcgtcacgaatggccgaataagtgcgaccatcttcagagcttcgtgtgactggcgaccatctttacccgaagtcagatagacaggaatcaccattggtagcagtgactaattaatgcactgttacaacacatgactgacaagtttcgaaaaccaagaataaggtactatcaatatcataagtacctaggatctaaggtatgtaggcagaccgtcatcatcaccttcaaacccccgacaggacaggcctcaatccccggcagtaggtacatactctatctccgggacttgacgacccaccattgcgattgccgcctcaatgccagaaggaacttttgtcctcccagtgctttgtcctgctactgtcattaccaagcaagccttaggagtcataagagtcatactgaaccttaggtacttgttgggcagagccatgtggcctacactcccaaactcaaaattactggtccgttcatgccttggatcatgtatctttccatttgccaatcataggcctcccggaactttcaagcaatagagaggtcagctcgatgctggacagggcagaccgtacttacacgtacctaggtagcctctctgtagaacctttgaccctcaaaaggttcatcaccaagttattgcgtagcatgacctagaatactgaaattagatcgcgcaagtagcaataattcgctatactatgtatgcggcaagtcgcatttcagaagccggttctgttcaaccacagtccaaccgtcgtcaatctggagatgcgtcacaggagccgcaggtgactgcacagcgatgcaccgtggtgatgacattgaatctgcctaggtataattacctacattttcaatgtctgtcttcaaaaatagaataaagtgccacttggcattcgacaattgttgtgttgaacaattgggagtatctacgtcgtgaatcatgttgcaagcaagaggtataggtaggtaccttacctgttgaagcagctagcgccctagaggcagcctctgatgtcgtcttgtcattttttgatccatctcaaacaagtctcaacaacgcatcccatgcaccatggagcttttcgcaacaggcttcaacgcctggaaccagctcactttcaccaaaggcagcccccaagaggccatcccagaggaaccagatgacctcttcggctttacaaaagttctctccgccacatccattgaacggccagtatcgcgcctcacttacaccatcggtaccttatatcaaatcacaacctatctcataccccatcacacctcccttttacgccctataaaagaccattaccgcctaaacctcaacaatcaaaccacaaactgacaaaagatttcccccccctccagtccgaaaattttcgact

SEQ ID NO: 4 - DNA, 2388 bp, Artificial Sequence
  Hygromycin B resistance marker
gttaacaagacacagccctataacttcgtataatgtatgctatacgaagttatataacggtgagactagcggccggtccccttatcccagctgttccacgttggcctgcccctcagttagcgctcaactcaatgcccctcactggcgaggcgagggcaaggatggaggggcagcatcgcctgagttggagcaaagcggcccggccgccatgggagcagcgaaccaacggagggatgccgtgctttgtcgtggctgctgtggccaatccgggcccttggttggctcacagagcgttgctgtgagaccatgagctattattgctaggtacagtatagagagaggagagagagagagagagagagagaggggaaaaaaggtgaggttgaagtgagaaaaaaaaaaaaaaaaaaaaatccaaccactgacggctgccggctctgccacccccctccctccaccccagaccacctgcacactcagcgcgcagcatcacctaatcttggctcgccttcccgcagctcaggttgttttttttttctctctccctcgtcgaagccgcccttgttcccttatttatttccctctccatccttgtctgcctttggtccatctgcccctttgtctgcatctcttttgcacgcatcgccttatcgtcgtctcttttttcactcacgggagcttgacgaagacctgactcgtgagcctcacctgctgatttctctccccccctcccgaccggcttgacttttgtttctcctccagtaccttatcgcgaagccggaagaacctcttaacctctagatgaaaaagcctgaactcaccgccacgtctgtcgagaagttcctgatcgaaaagttcgacagcgtctccgacctgatgcagctctcggagggcgaagaatctcgtgctttcagcttcgatgtaggagggcgtggatatgtcctgcgggtaaatagctgcgccgatggtttctacaaagatcgttatgtttatcggcactttgcatcggccgcgctcccgattccggaagtgcttgacattggggaattcagcgagagcctgacctattgcatctcccgccgtgcacagggtgtcacgttgcaagacctgcctgaaaccgaactgcccgctgttctgcagccggtcgcggaggccatggatgcgatcgctgcggccgatctcagccagacgagcgggttcggcccattcggaccgcaaggaatcggtcaatacactacatggcgtgatttcatatgcgcgattgctgatccccatgtgtatcactggcaaactgtgatggacgacaccgtcagtgcgtccgtcgcgcaggctctcgatgagctgatgctttgggccgaggactgccccgaagtccggcacctcgtgcacgcggatttcggctccaacaatgtcctgacggacaatggccgcataacagcggtcattgactggagcgaggcgatgttcggggattcccaatacgaggtcgccaacatcttcttctggaggccgtggttggcttgtatggagcagcagacgcgctacttcgagcggaggcacccggagcttgcaggatcgccgcggctccgggcgtatatgctccgcattggtcttgaccaactctatcagagcttggttgacggcaatttcgatgatgcagcttgggcgcagggtcgatgcgacgcaatcgtccgatccggagccgggactgtcgggcgtacacaaatcgcccgcagaagcgcggccgtctggaccgatggctgtgtagaagtactcgccgatagtggaaaccgacgccccagcactcgtccgagggcaaaggaatagatgcatggctttcgtgaccgggcttcaaacaatgatgtgcgatggtgtggttcccggttggcggagtctttgtctactttggttgtctgtcgcaggtcggtagaccgcaaatgagcaactgatggattgttgccagcgatactataattcacatggatggtctttgtcgatcagtagctagtgagagagagagaacatctatccacaatgtcgagtgtctattagacatactccgagaataaagtcaactgtgtctgtgatctaaagatcgattcggcagtcgagtagcgtataacaactccgagtaccagcgaaagcacgtcgtgacaggagcagggctttgccaactgcgcaaccttgcttgaatgaggatacacggggtgcaacatggctgtactgatccatcgcaaccaaaatttctgtttatagatcaagctggtagattccaattactccacctcttgcgcttctccatgacatgtaagtgcacgtggaaaccatacccaatataacttcgtataatgtatgctatacgaagttatagggctcttgtctgttaac

SEQ ID NO: 5 - DNA, 20 bp, Artificial Sequence
  SEQ1D5fw
gactctctatctgcatcaac

SEQ ID NO: 6 - DNA, 54 bp, Artificial Sequence
  SEQ1D5rv
tgacctggaaagctttcaatgtagaggtagactagtcaaagaagacatcacgac

SEQ ID NO: 7 - DNA, 55 bp, Artificial Sequence
  SEQ1D3fw
cgcatggtgggcgtcgtgatgtcttctttgactagtctacctctacattgaaagc

SEQ ID NO: 8 - DNA, 20 bp, Artificial Sequence
  SEQ1D3rv
gattacctgtcaagtctatg

SEQ ID NO: 9 - DNA, 32 bp, Artificial Sequence
  SEQ1Dnestfw
gacagtcctgcaggagtcactgcctttgaaag

SEQ ID NO: 10 - DNA, 33 bp, Artificial Sequence
  SEQ1Dnestrv
gacagtcctgcaggtgtaaggataaaggacgac

SEQ ID NO: 11 - DNA, 39 bp, Artificial Sequence
  LIC1fw
ctaggagttctgccttgggtttaaacgagagaaagactc

SEQ ID NO: 12 - DNA, 39 bp, Artificial Sequence
  LIC1rv
ctaggagtctttctctcgtttaaacccaaggcagaactc

SEQ ID NO: 13 - DNA, 37 bp, Artificial Sequence
  SEQ1DHygRfw
gttctgccttgggtttaacaagacacagccctataac

SEQ ID NO: 14 - DNA, 36 bp, Artificial Sequence
  SEQ1DHygRrv
gtctttctctcgtttaacagacaagagccctataac

SEQ ID NO: 15 - DNA, 19 bp, Artificial Sequence
  SEQ1DKO1fw
actctctatctgcatcaac

SEQ ID NO: 16 - DNA, 19 bp, Artificial Sequence
  SEQ1DKO1rv
gtagtgtattgaccgattc

SEQ ID NO: 17 - DNA, 20 bp, Artificial Sequence
  SEQ1DKO2fw
tgatgtgcttgatattgggc

SEQ ID NO: 18 - DNA, 20 bp, Artificial Sequence
  SEQ1DKO2rv
ctccatcgctcaactatgtg

SEQ ID NO: 19 - DNA, 21 bp, Artificial Sequence
  SEQ1MHygRfw
aacaagacacagccctataac

SEQ ID NO: 20 - DNA, 21 bp, Artificial Sequence
  SEQ1MHygRrv
aacagacaagagccctataac

SEQ ID NO: 21 - DNA, 19 bp, Artificial Sequence
  SEQ1M1KOfw
gatggctgtgtagaagtac

SEQ ID NO: 22 - DNA, 19 bp, Artificial Sequence
  SEQ1M1KOrv
atgaataggagtgtgtgtg

SEQ ID NO: 23 - DNA, 18 bp, Artificial Sequence
  SEQ1M1Seqfw
atactcgtcaactccatc

SEQ ID NO: 24 - DNA, 18 bp, Artificial Sequence
  SEQ1M1Seqrv
atcgctcaactatgtgac

SEQ ID NO: 25 - DNA, 20 bp, Artificial Sequence
  M1Seq-01
agcaagtcaaagtcatgagg

SEQ ID NO: 26 - DNA, 19 bp, Artificial Sequence
  SEQ1M2KOfw
gatggctgtgtagaagtac

SEQ ID NO: 27 - DNA, 19 bp, Artificial Sequence
  SEQ1M2KOrv
atgaataggagtgtgtgtg

SEQ ID NO: 28 - DNA, 20 bp, Artificial Sequence
  SEQ1M2Seqfw
gacagaagctcaaagattag

SEQ ID NO: 29 - DNA, 18 bp, Artificial Sequence
  SEQ1M2Seqrv
caagtcaaagtcatgagg

SEQ ID NO: 30 - DNA, 20 bp, Artificial Sequence
  M2Seq-01
cactctgtaaaggcaaaggg